European Patent Application EP 4 682 539 A1, published January 21, 2026. Title: Method for detecting misfolded alpha-synuclein protein in biological samples to determine the presence of synucleinopathies in an individual. Applicant: MODAG GmbH. The sequence listing filed with the application follows.

SEQUENCE LISTING (2 sequences)

SEQ ID NO: 1 - protein, 140 aa, human
MDVFMKGLSKAKEGVVAAAEKTKQGVAEAAGKTKEGVLYVGSKTKEGVVHGVATVAEKTKEQVTNVGGAVVTGVTAVAQKTVEGAGSIAAATGFVKKDQLGKNEEGAPQEGILEDMPVDPDNEAYEMPSEEGYQDYEPEA

SEQ ID NO: 2 - protein, 160 aa, synthetic construct
MGSSHHHHHHSSGLVPRGSHMDVFMKGLSKAKEGVVAAAEKTKQGVAEAAGKTKEGVLYVGSKTKEGVVHGVATVAEKTKEQVTNVGGAVVTGVTAVAQKTVEGAGSIAAATGFVKKDQLGKNEEGAPQEGILEDMPVDPDNEAYEMPSEEGYQDYEPEA